European Patent Specification EP 3 528 815 B1, published June 14, 2023. Title: Dérivés de la purine pour leur utilisation dans le traitement ou la prévention de maladies dues à une mutation non-sens. Applicant: MUSEUM NATIONAL D'HISTOIRE NATURELLE CENTRE NATIONAL DE LA RECHERCHE SCIENTIFIQUE UNIVERSITE LILLE 1, SCIENCES ET TECHNOLOGIES INSTITUT PASTEUR DE LILLE. The sequence listing filed with the application follows.

SEQUENCE LISTING (10 sequences)

SEQ ID NO: 1 - DNA, 19 bp, Artificial Sequence
  Primer
atgtgctcaagactggcgc

SEQ ID NO: 2 - DNA, 18 bp, Artificial Sequence
  Primer
gacagcatcaaatcatcc

SEQ ID NO: 3 - DNA, 20 bp, Artificial Sequence
  Primer
cattgacctcaactacatgg

SEQ ID NO: 4 - DNA, 19 bp, Artificial Sequence
  Primer
gccatgccagtgagcttcc

SEQ ID NO: 5 - DNA, 20 bp, Artificial Sequence
  Primer
ggaagaccatgtggacctgt

SEQ ID NO: 6 - DNA, 20 bp, Artificial Sequence
  Primer
gacaagtggggaggaggaag

SEQ ID NO: 7 - DNA, 20 bp, Artificial Sequence
  Primer
ggaggaggaggatgacatcg

SEQ ID NO: 8 - DNA, 20 bp, Artificial Sequence
  Primer
gcttgcagtcagtctcactc

SEQ ID NO: 9 - DNA, 20 bp, Artificial Sequence
  Primer
cagagctggaagtcgagtgt

SEQ ID NO: 10 - DNA, 20 bp, Artificial Sequence
  Primer
aggagtcccctcatgcaagt